European Patent Specification EP 3 810 283 B1, published June 14, 2023. Title: SOLID FORMS OF 3-((1R,3R)-1-(2,6-DIFLUORO-4-((1-(3-FLUOROPROPYL) AZETIDIN-3-YL)AMINO)PHENYL)-3-METHYL-1,3,4,9-TETRAHYDRO -2H-PYRIDO[3,4-B]INDOL-2-YL)-2,2-DIFLUOROPROPAN-1-OL AND PROCESSES FOR PREPARING FUSED TRICYCLIC COMPOUNDS COMPRISING A SUBSTITUTED PHENYL OR PYRIDINYL MOIETY, INCLUDING METHODS OF THEIR USE. Applicant: GENENTECH, INC. The sequence listing filed with the application follows.

SEQUENCE LISTING (4 sequences)

SEQ ID NO: 1 - protein, 457 aa, Artificial Sequence
  source: /note="Description of Artificial Sequence: Synthetic polypeptide"
MLKNDQLDQWDRDNFFHPSTHLAQHARGESANRVIKTASGVFIEDRDGTKLLDAFAGLFCVNVGYGRQEIAEAIADQARELAYYHSFVGHGTEASITLAKMILDRAPKNMSKVYFGLGGSDANETNVKLIWYYNNILGRPEKKKIISRWRGYHGSGLVTGSLTGLELFHKKFDLPVEQVIHTEAPYYFRREDLNQTEEQFVAHCVAELEALIEREGADTIAAFIGEPILGGGGIVPPPAGYWEAIQTVLNKHDILLVADEVVTGFGRLGTMFGSDHYGLEPDIITIAKGLTSAYAPLSGSIVSDKVWKVLEQGTDENGPIGHGWTYSAHPIGAAAGVANLKLLDELNLVSNAGEVGAYLNATMAEALSQHANVGDVRGEGLLCAVEFVKDRDSRTFFDAADKIGPQISAKLLEQDKIIARAMPQGDILGFAPPFCLTRAEADQVVEGTLRAVKAVLG

SEQ ID NO: 2 - protein, 457 aa, Artificial Sequence
  source: /note="Description of Artificial Sequence: Synthetic polypeptide"
MLKNDQLDQWDRDNFFHPSTHLAQHARGESANRVIKTASGVFIEDRDGTKLLDAFAGLWCVNVGYGRQEIAEAIADQARELAYYHSFVGHGTEASITLAKMILDRAPKNMSKVYFGLGGSDANETNVKLIWYYNNILGRPEKKKIISRWRGYHGSGLVTGSLTGLELFHKKFDLPVEQVIHTEAPYYFRREDLNQTEEQFVAHCVAELEALIEREGADTIAAFIGEPILGAGGIVPPPAGYWEAIQTVLNKHDILLVADEVVTGFGRLGTMFGSDHYGLEPDIITIAKGLTSAYAPLSGSIVSDKVWKVLEQGTDENGPIGHGWTYSAHPIGAAAGVANLKLLDELNLVSNAGEVGAYLNATMAEALSQHANVGDVRGEGLLCAVEFVKDRDSRTFFDAADKIGPQISAKLLEQDKIIARAMPQGDILGFAPPFCLTRAEADQVVEGTLRAVKAVLG

SEQ ID NO: 3 - protein, 457 aa, Artificial Sequence
  source: /note="Description of Artificial Sequence: Synthetic polypeptide"
MLKNDQLDQWDRDNFFHPSTHLAQHARGESANRVIKTASGVFIEDRDGTKLLDAFAGLFCVNVGYGRQEIAEAIADQARELAYYHAFVGHGTEASITLAKMILDRAPKNMSKVYFGLGGSDANETNVKLIWYYNNILGRPEKKKIISRWRGFHGSGLVTGSLTGLELFHKKFDLPVEQVIHTEAPYYFRREDLNQTEEQFVAHCVAELEALIEREGADTIAAFIGEPILGAGGMVPPPAGYWEAIQTVLNKHDILLVADEVVTGFGRLGTMFGSDHYGLEPDIITIAKGLTSAYAPLSGSIVSDKVWKVLEQGTDENGPIGHGWTYSAHPIGAAAGVANLKLLDELNLVSNAGEVGAYLNATMAEALSQHANVGDVRGEGLMCAVEFVKDRDSRTFFDAADKIGPQISAKLLEQDKIIARAMPQGDILGFAPPFCLTRAEADQVVEGTLRAVKAVLG

SEQ ID NO: 4 - protein, 464 aa, Artificial Sequence
  source: /note="Description of Artificial Sequence: Synthetic polypeptide"
MATITNHMPTAELQALDAAHHLHPFSANNALGEEGTRVITRARGVWLNDSALAQKLAELAGLWCVNIGYGRDELAEVAARQMRELPYYNTFFKTTHVPAIALAQKLAELAPGDLNHVFFAGGGSEANDTNIRMVRTYWQNKGQPEKTVIISRKNAYHGSTVASSALGGMAGMHAQSGLIPDVHHINQPNWWAEGGDMDPEEFGLARARELEEAILELGENRVAAFIAEPVQGAGGVIVAPDSYWPEIQRICDKYDILLIADEVVCGFGRTGNWFGTQTMGIRPHIMTIAKGLSSGYAPIGGSIVCDEVAHVIGKDEFNHGYTYSGHPVAAAVALENLRILEEENILDHVRNVAAPYLKEKWEALTDHPLVGEAKIVGMMASIALTPNKASRAKFASEPGTIGYICRERCFANNLIMRHVGDRMIISPPLVITPAEIDEMFVRIRKSLDEAQAEIEKQGLMKSAA